European Patent Application EP 4 483 951 A1, published January 1, 2025. Title: Single-domain antibody for inhibition of neutrophil elastase activity. Applicant: Université de Liège. Application EP. The sequence listing filed with the application follows.

SEQUENCE LISTING (22 sequences)

SEQ ID NO: 1 - protein, 8 aa, synthetic construct
GRTISLYR

SEQ ID NO: 2 - protein, 8 aa, synthetic construct
INWSGDMT

SEQ ID NO: 3 - protein, 16 aa, synthetic construct
TADPKLLPLADSSYGY

SEQ ID NO: 4 - protein, 123 aa, synthetic construct
QVQLQESGGGLVQAGGSLRLSCVVPGRTISLYRMGWFRQAPGKEREFVAGINWSGDMTDYVDSVKGRFTISRDNAKNTVYLEMNSLKPEDTAIYYCTADPKLLPLADSSYGYWGQGTQVTVSS

SEQ ID NO: 5 - DNA, 23 bp, synthetic construct
  source 1..23: mol_type = other DNA
gtcctggctgctcttctacaagg

SEQ ID NO: 6 - DNA, 23 bp, synthetic construct
  source 1..23: mol_type = other DNA
ggtacgtgctgttgaactgttcc

SEQ ID NO: 7 - DNA, 34 bp, synthetic construct
  source 1..34: mol_type = other DNA
ctagtgcggccgctgaggagacggtgacctgggt

SEQ ID NO: 8 - DNA, 29 bp, synthetic construct
  source 1..29: mol_type = other DNA
gatgtgcagctgcaggagtctggrggagg

SEQ ID NO: 9 - DNA, 20 bp, synthetic construct
  source 1..20: mol_type = other DNA
ttatgcttccggctcgtatg

SEQ ID NO: 10 - DNA, 18 bp, synthetic construct
  source 1..18: mol_type = other DNA
ccacagacagccctcata

SEQ ID NO: 11 - protein, 29 aa, synthetic construct
TSVHQETKKMCTASIPPQCYYNYEWHVDV

SEQ ID NO: 12 - protein, 11 aa, synthetic construct
MCTASIPPQCY

SEQ ID NO: 13 - protein, 267 aa, Homo sapiens
MTLGRRLACLFLACVLPALLLGGTALASEIVGGRRARPHAWPFMVSLQLRGGHFCGATLIAPNFVMSAAHCVANVNVRAVRVVLGAHNLSRREPTRQVFAVQRIFENGYDPVNLLNDIVILQLNGSATINANVQVAQLPAQGRRLGNGVQCLAMGWGLLGRNRGIASVLQELNVTVVTSLCRRSNVCTLVRGRQAGVCFGDSGSPLVCNGLIHGIASFVRGGCASGLYPDAFAPVAQFVNWIDSIIQRSEDNPCPHPRDPDPASRTH

SEQ ID NO: 14 - protein, 218 aa, Homo sapiens [sequence omitted]

SEQ ID NO: 15 - protein, 124 aa, synthetic construct
QVQLQESGGGLVQPGGSLRLSCAASGFTLDYHAIGWFRQAPGKEREGVSCISSSGGRADYADSVKGRFTISRDNAKNTVYLQMNSLKPEDTAVYYCATRCAVVGGTYYYGMDYWGKGTQVTVSS

SEQ ID NO: 16 - protein, 14 aa, synthetic construct
SPSTPPTPSPSTPP

SEQ ID NO: 17 - protein, 25 aa, synthetic construct
QVQLQESGGGLVQAGGSLRLSCVVP

SEQ ID NO: 18 - protein, 17 aa, synthetic construct
MGWFRQAPGKEREFVAG

SEQ ID NO: 19 - protein, 38 aa, synthetic construct
DYVDSVKGRFTISRDNAKNTVYLEMNSLKPEDTAIYYC

SEQ ID NO: 20 - protein, 11 aa, synthetic construct
WGQGTQVTVSS

SEQ ID NO: 21 - protein, 137 aa, synthetic construct
QVQLQESGGGLVQPGGSLRLSCAASGFTLDYHAIGWFRQAPGKEREGVSCISSSGGRADYADSVKGRFTISRDNAKNTVYLQMNSLKPEDTAVYYCATRCAVVGGTYYYGMDYWGKGTQVTVSSAAAYPYDVPDYGS

SEQ ID NO: 22 - protein, 15 aa, synthetic construct
SPSTPPTPSPSTPPC